European Patent Specification EP 3 463 396 B1, published April 8, 2026. Title: CHIMERIC ANTIGEN RECEPTOR AND CAR-T CELLS THAT BIND BCMA. Applicant: MAX-DELBRÜCK-CENTRUM FÜR MOLEKULARE MEDIZIN Humboldt-Universität zu Berlin. The sequence listing filed with the application follows.

SEQUENCE LISTING (94 sequences)

SEQ ID NO: 1 - protein, 8 aa, Artificial Sequence
  CDR
GFTFSRYW

SEQ ID NO: 2 - protein, 8 aa, Artificial Sequence
  CDR
INPSSSTI

SEQ ID NO: 3 - protein, 13 aa, Artificial Sequence
  CDR
ASLYYDYGDAYDY

SEQ ID NO: 4 - protein, 6 aa, Artificial Sequence
  CDR
QSVESN

SEQ ID NO: 5 - protein, 4 aa, Artificial Sequence
  CDR
  misc_feature (4)..(4): Xaa can be any naturally occurring amino acid
SASX

SEQ ID NO: 6 - protein, 9 aa, Artificial Sequence
  CDR
QQYNNYPLT

SEQ ID NO: 7 - protein, 8 aa, Artificial Sequence
  CDR
  misc_feature (4)..(5): Xaa can be any naturally occurring amino acid
INPXXSTI

SEQ ID NO: 8 - protein, 13 aa, Artificial Sequence
  CDR
  misc_feature (5)..(5): Xaa can be any naturally occurring amino acid
  misc_feature (11)..(11): Xaa can be any naturally occurring amino acid
ASLYXDYGDAXDY

SEQ ID NO: 9 - protein, 6 aa, Artificial Sequence
  CDR
  misc_feature (4)..(5): Xaa can be any naturally occurring amino acid
QSVXXN

SEQ ID NO: 10 - protein, 11 aa, Artificial Sequence
  CDR
QQYNNYPLTFG

SEQ ID NO: 11 - protein, 120 aa, Artificial Sequence
  VH
EVQLVESGGGLVQPGGSLRLSCAASGFTFSRYWFSWVRQAPGKGLVWVGEINPSSSTINYAPSLKDKFTISRDNAKNTLYLQMNSLRAEDTAVYYCASLYYDYGDAYDYWGQGTLVTVSS

SEQ ID NO: 12 - protein, 107 aa, Artificial Sequence
  VL
EIVMTQSPATLSVSPGERATLSCKASQSVESNVAWYQQKPGQAPRALIYSASLRFSGIPARFSGSGSGTEFTLTISSLQSEDFAVYYCQQYNNYPLTFGAGTKLELK

SEQ ID NO: 13 - protein, 18 aa, Artificial Sequence
  linker
GSTSGSGKPGSGEGSTKG

SEQ ID NO: 14 - protein, 17 aa, Artificial Sequence
  linker
SSGGGGSGGGGSGGGGS

SEQ ID NO: 15 - protein, 234 aa, Artificial Sequence
  spacer
PAEPKSPDKTHTCPPCPAPPVAGPSVFLFPPKPKDTLMIARTPEVTCVVVDVSHEDPEVKFNWYVDGVEVHNAKTKPREEQYNSTYRVVSVLTVLHQDWLNGKEYKCKVSNKALPAPIEKTISKAKGQPREPQVYTLPPSRDELTKNQVSLTCLVKGFYPSDIAVEWESNGQPENNYKTTPPVLDSDGSFFLYSKLTVDKSRWQQGNVFSCSVMHEALHNHYTQKSLSLSPGKK

SEQ ID NO: 16 - protein, 235 aa, Artificial Sequence
  spacer
PAEPKSPDKTHTCPPCPAPPVAGPSVFLFPPKPKDTLMIARTPEVTCVVVDVSHEDPEVKFNWYVDGVEVHNAKTKPREEQYNSTYRVVSVLTVLHQDWLNGKEYKCKVSNKALPAPIEKTISKAKGQPREPQVYTLPPSRDELTKNQVSLTCLVKGFYPSDIAVEWESNGQPENNYKTTPPVLDSDGSFFLYSKLTVDKSRWQQGNVFSCSVMHEALHNHYTQKSLSSLSPGKK

SEQ ID NO: 17 - protein, 229 aa, Artificial Sequence
  spacer
ESKYGPPCPPCPAPEFEGGPSVFLFPPKPKDTLMISRTPEVTCVVVDVSQEDPEVQFNWYVDGVEVHNAKTKPREEQFNSTYRVVSVLTVLHQDWLNGKEYKCKVSNKGLPSSIEKTISKAKGQPREPQVYTLPPSQEEMTKNQVSLTCLVKGFYPSDIAVEWESNGQPENNYKTTPPVLDSDGSFFLYSRLTVDKSRWQEGNVFSCSVMHEALHNHYTQKSLSLSLGK

SEQ ID NO: 18 - protein, 119 aa, Artificial Sequence
  spacer
ESKYGPPCPPCPGQPREPQVYTLPPSQEEMTKNQVSLTCLVKGFYPSDIAVEWESNGQPENNYKTTPPVLDSDGSFFLYSRLTVDKSRWQEGNVFSCSVMHEALHNHYTQKSLSLSLGK

SEQ ID NO: 19 - protein, 12 aa, Artificial Sequence
  spacer
ESKYGPPCPPCP

SEQ ID NO: 20 - protein, 24 aa, Artificial Sequence
  transmembrane
IYIWAPLAGTCGVLLLSLVITLYC

SEQ ID NO: 21 - protein, 27 aa, Artificial Sequence
  transmembrane
FWVLVVVGGVLACYSLLVTVAFIIFWV

SEQ ID NO: 22 - protein, 42 aa, Artificial Sequence
  intracellular
KRGRKKLLYIFKQPFMRPVQTTQEEDGCSCRFPEEEEGGCEL

SEQ ID NO: 23 - protein, 41 aa, Artificial Sequence
  intracellular
RSKRSRLLHSDYMNMTPRRPGPTRKHYQPYAPPRDFAAYRS

SEQ ID NO: 24 - protein, 113 aa, Artificial Sequence
  intracellular
LRVKFSRSADAPAYQQGQNQLYNELNLGRREEYDVLDKRRGRDPEMGGKPRRKNPQEGLYNELQKDKMAEAYSEIGMKGERRRGKGHDGLYQGLSTATKDTYDALHMQALPPR

SEQ ID NO: 25 - protein, 5 aa, Artificial Sequence
  CDR
RYWFS

SEQ ID NO: 26 - protein, 18 aa, Artificial Sequence
  CDR
EINPSSSTINYAPSLKDK

SEQ ID NO: 27 - protein, 13 aa, Artificial Sequence
  CDR
SLYYDYGDAYDYW

SEQ ID NO: 28 - protein, 11 aa, Artificial Sequence
  CDR
KASQSVESNVA

SEQ ID NO: 29 - protein, 7 aa, Artificial Sequence
  CDR
SASLRFS

SEQ ID NO: 30 - protein, 11 aa, Artificial Sequence
  CDR
QQYNNYPLTFG

SEQ ID NO: 31 - protein, 53 aa, Homo sapiens
MAGQCSQNEYFDSLLHACIPCQLRCSSNTPPLTCQRYCNASVTNSVKGTNALE

SEQ ID NO: 32 - protein, 56 aa, Homo sapiens
MLQMAGQCSQNEYFDSLLHACIPCQLRCSSNTPPLTCQRYCNASVTNSVKGTNALE

SEQ ID NO: 33 - protein, 20 aa, Homo sapiens
YFDSLLHACIPCQLRCSSNT

SEQ ID NO: 34 - protein, 5 aa, Artificial Sequence
  CDR
  misc_feature (4)..(4): Xaa can be any naturally occurring amino acid
RYWXS

SEQ ID NO: 35 - protein, 18 aa, Artificial Sequence
  CDR
  misc_feature (5)..(6): Xaa can be any naturally occurring amino acid
EINPXXSTINYAPSLKDK

SEQ ID NO: 36 - protein, 13 aa, Artificial Sequence
  CDR
  misc_feature (4)..(4): Xaa can be any naturally occurring amino acid
  misc_feature (10)..(10): Xaa can be any naturally occurring amino acid
SLYXDYGDAXDYW

SEQ ID NO: 37 - protein, 11 aa, Artificial Sequence
  CDR
  misc_feature (7)..(8): Xaa can be any naturally occurring amino acid
KASQSVXXNVA

SEQ ID NO: 38 - protein, 120 aa, Artificial
  mouse Ab
QVQLQQSGGGLVQPGGSLKLSCAASGIDFSRYWMSWVRRAPGKGLEWIGEINPDSSTINYAPSLKDKFIISRDNAKNTLYLQMSKVRSEDTALYYCASLYYDYGDAMDYWGQGTSVTVSS

SEQ ID NO: 39 - protein, 120 aa, Artificial Sequence
  Ab
EVQLVESGGGLVQPGGSLRLSCAASGFTFDDYWMSWVRQAPGKGLEWVGEINPDSSTINYAPSLKGRFTISRDNAKNTLYLQMNSLRAEDTAVYYCASLYYDYGDAMDYWGQGTLVTVSS

SEQ ID NO: 40 - protein, 120 aa, Artificial Sequence
  VH
EVQLVESGGGLVQPGGSLRLSCAASGFTFSRYWMSWVRQAPGKGLVWVGEINPDSSTINYAPSLKDKFTISRDNAKNTLYLQMNSLRAEDTAVYYCASLYYDYGDAMDYWGQGTLVTVSS

SEQ ID NO: 41 - protein, 120 aa, Artificial Sequence
  VH
  misc_feature (34)..(34): Xaa can be any naturally occurring amino acid
  misc_feature (54)..(55): Xaa can be any naturally occurring amino acid
  misc_feature (101)..(101): Xaa can be any naturally occurring amino acid
  misc_feature (107)..(107): Xaa can be any naturally occurring amino acid
EVQLVESGGGLVQPGGSLRLSCAASGFTFSRYWXSWVRQAPGKGLVWVGEINPXXSTINYAPSLKDKFTISRDNAKNTLYLQMNSLRAEDTAVYYCASLYXDYGDAXDYWGQGTLVTVSS

SEQ ID NO: 42 - protein, 120 aa, Artificial Sequence
  VH
  misc_feature (33)..(33): Xaa can be any naturally occurring amino acid
  misc_feature (35)..(35): Xaa can be any naturally occurring amino acid
  misc_feature (47)..(47): Xaa can be any naturally occurring amino acid
  misc_feature (50)..(50): Xaa can be any naturally occurring amino acid
  misc_feature (99)..(101): Xaa can be any naturally occurring amino acid
  misc_feature (106)..(106): Xaa can be any naturally occurring amino acid
EVQLVESGGGLVQPGGSLRLSCAASGFTFSRYXMXWVRQAPGKGLVXVGXINPDSSTINYAPSLKDKFTISRDNAKNTLYLQMNSLRAEDTAVYYCASXXXDYGDXMDYWGQGTLVTVSS

SEQ ID NO: 43 - protein, 120 aa, Artificial Sequence
  VH
EVQLVESGGGLVQPGGSLRLSCAASGFTFSRYWISWVRQAPGKGLVWVGEINPNSSTINYAPSLKDKFTISRDNAKNTLYLQMNSLRAEDTAVYYCASLYYDYGDAYDYWGQGTLVTVSS

SEQ ID NO: 44 - protein, 120 aa, Artificial Sequence
  VH
EVQLVESGGGLVQPGGSLRLSCAASGFTFSRYWFSWVRQAPGKGLVWVGEINPNSSTINYAPSLKDKFTISRDNAKNTLYLQMNSLRAEDTAVYYCASLYYDYGDAYDYWGQGTLVTVSS

SEQ ID NO: 45 - protein, 120 aa, Artificial Sequence
  VH
EVQLVESGGGLVQPGGSLRLSCAASGFTFSRYWISWVRQAPGKGLVWVGEINPSSSTINYAPSLKDKFTISRDNAKNTLYLQMNSLRAEDTAVYYCASLYYDYGDAYDYWGQGTLVTVSS

SEQ ID NO: 46 - protein, 120 aa, Artificial Sequence; identical to SEQ ID NO: 11
  VH

SEQ ID NO: 47 - protein, 108 aa, Artificial Sequence
  VL
DIVMTQSQRFMTTSVGDRVSVTCKASQSVDSNVAWYQQKPRQSPKALIFSASLRFSGVPARFTGSGSGTDFTLTISNLQSEDLAEYFCQQYNNYPLTFGAGTKLELKR

SEQ ID NO: 48 - protein, 108 aa, Artificial Sequence
  VL
DIVMTQSPATLSVSVGDEVTLTCKASQSVDSNVAWYQQKPGQAPKLLIYSDDLRFSGVPARFSGSGSGTDFTLTISSLQSEDFAVYYCQQYNNYPLTFGAGTKLELKR

SEQ ID NO: 49 - protein, 108 aa, Artificial Sequence
  VL
EIVMTQSPATLSVSPGERATLSCKASQSVDSNVAWYQQKPGQAPRALIYSASLRFSGIPARFSGSGSGTEFTLTISSLQSEDFAVYYCQQYNNYPLTFGAGTKLELKR

SEQ ID NO: 50 - protein, 108 aa, Artificial Sequence
  VL
  misc_feature (30)..(31): Xaa can be any naturally occurring amino acid
EIVMTQSPATLSVSPGERATLSCKASQSVXXNVAWYQQKPGQAPRALIYSASLRFSGIPARFSGSGSGTEFTLTISSLQSEDFAVYYCQQYNNYPLTFGAGTKLELKR

SEQ ID NO: 51 - protein, 108 aa, Artificial Sequence
  VL
  misc_feature (31)..(32): Xaa can be any naturally occurring amino acid
  misc_feature (34)..(34): Xaa can be any naturally occurring amino acid
  misc_feature (36)..(36): Xaa can be any naturally occurring amino acid
  misc_feature (49)..(50): Xaa can be any naturally occurring amino acid
  misc_feature (52)..(53): Xaa can be any naturally occurring amino acid
  misc_feature (55)..(55): Xaa can be any naturally occurring amino acid
  misc_feature (66)..(67): Xaa can be any naturally occurring amino acid
  misc_feature (89)..(89): Xaa can be any naturally occurring amino acid
  misc_feature (91)..(91): Xaa can be any naturally occurring amino acid
  misc_feature (94)..(94): Xaa can be any naturally occurring amino acid
  misc_feature (96)..(96): Xaa can be any naturally occurring amino acid
EIVMTQSPATLSVSPGERATLSCKASQSVDXXVXWXQQKPGQAPRALIXXAXXRXSGIPARFSGSXXGTEFTLTISSLQSEDFAVYYCXQXNNXPXTFGAGTKLELKR

SEQ ID NO: 52 - protein, 108 aa, Artificial Sequence
  VL
EIVMTQSPATLSVSPGERATLSCKASQSVESNVAWYQQKPGQAPRALIYSASLRFSGIPARFSGSGSGTEFTLTISSLQSEDFAVYYCQQYNNYPLTFGAGTKLELKR

SEQ ID NO: 53 - protein, 120 aa, Artificial Sequence
  VH
  misc_feature (1)..(1): Xaa can be any naturally occurring amino acid
  misc_feature (5)..(6): Xaa can be any naturally occurring amino acid
  misc_feature (19)..(19): Xaa can be any naturally occurring amino acid
  misc_feature (27)..(28): Xaa can be any naturally occurring amino acid
  misc_feature (30)..(31): Xaa can be any naturally occurring amino acid
  misc_feature (39)..(39): Xaa can be any naturally occurring amino acid
  misc_feature (48)..(48): Xaa can be any naturally occurring amino acid
  misc_feature (66)..(67): Xaa can be any naturally occurring amino acid
  misc_feature (69)..(69): Xaa can be any naturally occurring amino acid
  misc_feature (84)..(86): Xaa can be any naturally occurring amino acid
  misc_feature (88)..(88): Xaa can be any naturally occurring amino acid
  misc_feature (93)..(93): Xaa can be any naturally occurring amino acid
  misc_feature (115)..(115): Xaa can be any naturally occurring amino acid
XVQLXXSGGGLVQPGGSLXLSCAASGXXFXXYWZSWVRXAPGKGLEWXGEINPZSSTINYAPSLKXXFXISRDNAKNTLYLQMXXXRXEDTAXYYCASLYYDYGDAZDYWGQGTXVTVSS

SEQ ID NO: 54 - protein, 108 aa, Artificial Sequence
  VL
  misc_feature (8)..(13): Xaa can be any naturally occurring amino acid
  misc_feature (18)..(18): Xaa can be any naturally occurring amino acid
  misc_feature (20)..(21): Xaa can be any naturally occurring amino acid
  misc_feature (41)..(41): Xaa can be any naturally occurring amino acid
  misc_feature (43)..(43): Xaa can be any naturally occurring amino acid
  misc_feature (46)..(46): Xaa can be any naturally occurring amino acid
  misc_feature (49)..(49): Xaa can be any naturally occurring amino acid
  misc_feature (51)..(52): Xaa can be any naturally occurring amino acid
  misc_feature (63)..(63): Xaa can be any naturally occurring amino acid
  misc_feature (77)..(77): Xaa can be any naturally occurring amino acid
  misc_feature (83)..(83): Xaa can be any naturally occurring amino acid
  misc_feature (85)..(85): Xaa can be any naturally occurring amino acid
  misc_feature (87)..(87): Xaa can be any naturally occurring amino acid
DIVMTQSXXXXXXSVGDXVXXTCKASQSVESNVAWYQQKPXQXPKXLIXSXXLRFSGVPARFXGSGSGTDFTLTISXLQSEDXAXYXCQQYNNYPLTFGAGTKLELKR

SEQ ID NO: 55 - protein, 21 aa, Artificial Sequence
  leader
MDFQVQIFSFLLISASVIMSR

SEQ ID NO: 56 - protein, 21 aa, Artificial Sequence
  leader
MLLLVTSLLLCELPHPAFLLI

SEQ ID NO: 57 - protein, 684 aa, Artificial Sequence
  construct
MDFQVQIFSFLLISASVIMSREVQLVESGGGLVQPGGSLRLSCAASGFTFSRYWFSWVRQAPGKGLVWVGEINPSSSTINYAPSLKDKFTISRDNAKNTLYLQMNSLRAEDTAVYYCASLYYDYGDAYDYWGQGTLVTVSSGSTSGSGKPGSGEGSTKGEIVMTQSPATLSVSPGERATLSCKASQSVESNVAWYQQKPGQAPRALIYSASLRFSGIPARFSGSGSGTEFTLTISSLQSEDFAVYYCQQYNNYPLTFGAGTKLELKPAEPKSPDKTHTCPPCPAPPVAGPSVFLFPPKPKDTLMIARTPEVTCVVVDVSHEDPEVKFNWYVDGVEVHNAKTKPREEQYNSTYRVVSVLTVLHQDWLNGKEYKCKVSNKALPAPIEKTISKAKGQPREPQVYTLPPSRDELTKNQVSLTCLVKGFYPSDIAVEWESNGQPENNYKTTPPVLDSDGSFFLYSKLTVDKSRWQQGNVFSCSVMHEALHNHYTQKSLSLSPGKKDPKFWVLVVVGGVLACYSLLVTVAFIIFWVRSKRSRLLHSDYMNMTPRRPGPTRKHYQPYAPPRDFAAYRSLRVKFSRSADAPAYQQGQNQLYNELNLGRREEYDVLDKRRGRDPEMGGKPRRKNPQEGLYNELQKDKMAEAYSEIGMKGERRRGKGHDGLYQGLSTATKDTYDALHMQALPPR

SEQ ID NO: 58 - protein, 684 aa, Artificial Sequence
  construct
MDFQVQIFSFLLISASVIMSREIVMTQSPATLSVSPGERATLSCKASQSVESNVAWYQQKPGQAPRALIYSASLRFSGIPARFSGSGSGTEFTLTISSLQSEDFAVYYCQQYNNYPLTFGAGTKLELKGSTSGSGKPGSGEGSTKGEVQLVESGGGLVQPGGSLRLSCAASGFTFSRYWFSWVRQAPGKGLVWVGEINPSSSTINYAPSLKDKFTISRDNAKNTLYLQMNSLRAEDTAVYYCASLYYDYGDAYDYWGQGTLVTVSSPAEPKSPDKTHTCPPCPAPPVAGPSVFLFPPKPKDTLMIARTPEVTCVVVDVSHEDPEVKFNWYVDGVEVHNAKTKPREEQYNSTYRVVSVLTVLHQDWLNGKEYKCKVSNKALPAPIEKTISKAKGQPREPQVYTLPPSRDELTKNQVSLTCLVKGFYPSDIAVEWESNGQPENNYKTTPPVLDSDGSFFLYSKLTVDKSRWQQGNVFSCSVMHEALHNHYTQKSLSLSPGKKDPKFWVLVVVGGVLACYSLLVTVAFIIFWVRSKRSRLLHSDYMNMTPRRPGPTRKHYQPYAPPRDFAAYRSLRVKFSRSADAPAYQQGQNQLYNELNLGRREEYDVLDKRRGRDPEMGGKPRRKNPQEGLYNELQKDKMAEAYSEIGMKGERRRGKGHDGLYQGLSTATKDTYDALHMQALPPR

SEQ ID NO: 59 - protein, 684 aa, Artificial Sequence; identical to SEQ ID NO: 57
  construct

SEQ ID NO: 60 - protein, 676 aa, Artificial Sequence
  construct
MDFQVQIFSFLLISASVIMSREVQLVESGGGLVQPGGSLRLSCAASGFTFSRYWFSWVRQAPGKGLVWVGEINPSSSTINYAPSLKDKFTISRDNAKNTLYLQMNSLRAEDTAVYYCASLYYDYGDAYDYWGQGTLVTVSSGSTSGSGKPGSGEGSTKGEIVMTQSPATLSVSPGERATLSCKASQSVESNVAWYQQKPGQAPRALIYSASLRFSGIPARFSGSGSGTEFTLTISSLQSEDFAVYYCQQYNNYPLTFGAGTKLELKESKYGPPCPPCPAPEFEGGPSVFLFPPKPKDTLMISRTPEVTCVVVDVSQEDPEVQFNWYVDGVEVHNAKTKPREEQFNSTYRVVSVLTVLHQDWLNGKEYKCKVSNKGLPSSIEKTISKAKGQPREPQVYTLPPSQEEMTKNQVSLTCLVKGFYPSDIAVEWESNGQPENNYKTTPPVLDSDGSFFLYSRLTVDKSRWQEGNVFSCSVMHEALHNHYTQKSLSLSLGKFWVLVVVGGVLACYSLLVTVAFIIFWVRSKRSRLLHSDYMNMTPRRPGPTRKHYQPYAPPRDFAAYRSLRVKFSRSADAPAYQQGQNQLYNELNLGRREEYDVLDKRRGRDPEMGGKPRRKNPQEGLYNELQKDKMAEAYSEIGMKGERRRGKGHDGLYQGLSTATKDTYDALHMQALPPR

SEQ ID NO: 61 - protein, 566 aa, Artificial Sequence
  construct
MDFQVQIFSFLLISASVIMSREVQLVESGGGLVQPGGSLRLSCAASGFTFSRYWFSWVRQAPGKGLVWVGEINPSSSTINYAPSLKDKFTISRDNAKNTLYLQMNSLRAEDTAVYYCASLYYDYGDAYDYWGQGTLVTVSSGSTSGSGKPGSGEGSTKGEIVMTQSPATLSVSPGERATLSCKASQSVESNVAWYQQKPGQAPRALIYSASLRFSGIPARFSGSGSGTEFTLTISSLQSEDFAVYYCQQYNNYPLTFGAGTKLELKESKYGPPCPPCPGQPREPQVYTLPPSQEEMTKNQVSLTCLVKGFYPSDIAVEWESNGQPENNYKTTPPVLDSDGSFFLYSRLTVDKSRWQEGNVFSCSVMHEALHNHYTQKSLSLSLGKFWVLVVVGGVLACYSLLVTVAFIIFWVRSKRSRLLHSDYMNMTPRRPGPTRKHYQPYAPPRDFAAYRSLRVKFSRSADAPAYQQGQNQLYNELNLGRREEYDVLDKRRGRDPEMGGKPRRKNPQEGLYNELQKDKMAEAYSEIGMKGERRRGKGHDGLYQGLSTATKDTYDALHMQALPPR

SEQ ID NO: 62 - protein, 459 aa, Artificial Sequence
  construct
MDFQVQIFSFLLISASVIMSREVQLVESGGGLVQPGGSLRLSCAASGFTFSRYWFSWVRQAPGKGLVWVGEINPSSSTINYAPSLKDKFTISRDNAKNTLYLQMNSLRAEDTAVYYCASLYYDYGDAYDYWGQGTLVTVSSGSTSGSGKPGSGEGSTKGEIVMTQSPATLSVSPGERATLSCKASQSVESNVAWYQQKPGQAPRALIYSASLRFSGIPARFSGSGSGTEFTLTISSLQSEDFAVYYCQQYNNYPLTFGAGTKLELKESKYGPPCPPCPFWVLVVVGGVLACYSLLVTVAFIIFWVRSKRSRLLHSDYMNMTPRRPGPTRKHYQPYAPPRDFAAYRSLRVKFSRSADAPAYQQGQNQLYNELNLGRREEYDVLDKRRGRDPEMGGKPRRKNPQEGLYNELQKDKMAEAYSEIGMKGERRRGKGHDGLYQGLSTATKDTYDALHMQALPPR

SEQ ID NO: 63 - protein, 680 aa, Artificial Sequence
  construct
MDFQVQIFSFLLISASVIMSREVQLVESGGGLVQPGGSLRLSCAASGFTFSRYWFSWVRQAPGKGLVWVGEINPSSSTINYAPSLKDKFTISRDNAKNTLYLQMNSLRAEDTAVYYCASLYYDYGDAYDYWGQGTLVTVSSGSTSGSGKPGSGEGSTKGEIVMTQSPATLSVSPGERATLSCKASQSVESNVAWYQQKPGQAPRALIYSASLRFSGIPARFSGSGSGTEFTLTISSLQSEDFAVYYCQQYNNYPLTFGAGTKLELKPAEPKSPDKTHTCPPCPAPPVAGPSVFLFPPKPKDTLMIARTPEVTCVVVDVSHEDPEVKFNWYVDGVEVHNAKTKPREEQYNSTYRVVSVLTVLHQDWLNGKEYKCKVSNKALPAPIEKTISKAKGQPREPQVYTLPPSRDELTKNQVSLTCLVKGFYPSDIAVEWESNGQPENNYKTTPPVLDSDGSFFLYSKLTVDKSRWQQGNVFSCSVMHEALHNHYTQKSLSSLSPGKKIYIWAPLAGTCGVLLLSLVITLYCKRGRKKLLYIFKQPFMRPVQTTQEEDGCSCRFPEEEEGGCELLRVKFSRSADAPAYQQGQNQLYNELNLGRREEYDVLDKRRGRDPEMGGKPRRKNPQEGLYNELQKDKMAEAYSEIGMKGERRRGKGHDGLYQGLSTATKDTYDALHMQALPPR

SEQ ID NO: 64 - protein, 680 aa, Artificial Sequence
  construct
MDFQVQIFSFLLISASVIMSREIVMTQSPATLSVSPGERATLSCKASQSVESNVAWYQQKPGQAPRALIYSASLRFSGIPARFSGSGSGTEFTLTISSLQSEDFAVYYCQQYNNYPLTFGAGTKLELKGSTSGSGKPGSGEGSTKGEVQLVESGGGLVQPGGSLRLSCAASGFTFSRYWFSWVRQAPGKGLVWVGEINPSSSTINYAPSLKDKFTISRDNAKNTLYLQMNSLRAEDTAVYYCASLYYDYGDAYDYWGQGTLVTVSSPAEPKSPDKTHTCPPCPAPPVAGPSVFLFPPKPKDTLMIARTPEVTCVVVDVSHEDPEVKFNWYVDGVEVHNAKTKPREEQYNSTYRVVSVLTVLHQDWLNGKEYKCKVSNKALPAPIEKTISKAKGQPREPQVYTLPPSRDELTKNQVSLTCLVKGFYPSDIAVEWESNGQPENNYKTTPPVLDSDGSFFLYSKLTVDKSRWQQGNVFSCSVMHEALHNHYTQKSLSSLSPGKKIYIWAPLAGTCGVLLLSLVITLYCKRGRKKLLYIFKQPFMRPVQTTQEEDGCSCRFPEEEEGGCELLRVKFSRSADAPAYQQGQNQLYNELNLGRREEYDVLDKRRGRDPEMGGKPRRKNPQEGLYNELQKDKMAEAYSEIGMKGERRRGKGHDGLYQGLSTATKDTYDALHMQALPPR

SEQ ID NO: 65 - protein, 680 aa, Artificial Sequence; identical to SEQ ID NO: 63
  construct

SEQ ID NO: 66 - DNA, 360 bp, Artificial Sequence
  VH
gaggtgcagctggtggaatctggcggaggactggtgcagcctggcggctctctgagactgtcttgtgccgccagcggcttcaccttcagccggtactggtttagctgggtgcgccaggcccctggcaagggactcgtgtgggtgggagagatcaaccccagcagcagcaccatcaactacgcccccagcctgaaggacaagttcaccatcagcagagacaacgccaagaacaccctgtacctgcagatgaacagcctgcgggccgaggacaccgccgtgtactattgtgccagcctgtactacgactacggcgacgcctacgattactggggccagggcacactggtgactgttagctcc

SEQ ID NO: 67 - DNA, 321 bp, Artificial Sequence
  VL
gagatcgtgatgacacagagccctgccaccctgagcgtgtccccaggcgaaagagctaccctgagctgcaaggccagccagagcgtggaaagcaacgtggcctggtatcagcagaagcccggacaggctcctcgggccctgatctacagcgccagcctgagattcagcggcatccccgccaggtttagcggctctggcagcggcaccgagttcaccctgacaatcagcagcctgcagagcgaggactttgccgtgtattactgccagcagtacaacaactaccccctgaccttcggagccggcaccaagctggagctgaag

SEQ ID NO: 68 - DNA, 360 bp, Artificial Sequence
  VH
gaagtgcagctggtcgaatctggaggaggcctggttcagcctggtggcagccttaggctctcttgtgcagcctctggctttaccttctcacggtattggttcagctgggtgagacaggctccagggaaaggtctggtgtgggtaggggagataaaccccagcagcagcacgatcaactatgctccgtcactgaaagacaagttcaccatttcccgcgataatgccaagaacactctctacttgcagatgaattcccttcgagccgaggatacagcggtgtactactgcgccagtctgtactacgactatggggacgcatacgactattggggacaaggcacactggtgactgttagctcc

SEQ ID NO: 69 - DNA, 321 bp, Artificial Sequence
  VL
gagatcgtgatgacccagtctcctgctaccctgagcgtttctcccggtgaaagggccacactcagctgcaaagcctctcaaagcgtggagagcaatgtcgcctggtatcagcagaaacctggccaagctccgagagcactgatctattccgcgtcattgcgcttttccggcataccagcacggtttagtggctcagggagtgggactgagttcactctgacgattagctcccttcagtcagaggatttcgccgtgtactactgtcagcagtacaacaactatcccctcacattcggagctggaaccaagctggaactgaag

SEQ ID NO: 70 - DNA, 63 bp, Artificial Sequence
  leader
atggatttccaggtgcagatcttcagcttcctgctgatctccgccagcgtgatcatgagccgc

SEQ ID NO: 71 - DNA, 63 bp, Artificial Sequence
  leader
atgcttctcctggtgacaagccttctgctctgtgagttaccacacccagcattcctcctgatc

SEQ ID NO: 72 - DNA, 54 bp, Artificial Sequence
  linker
ggcagcaccagcggctccggcaagcctggctctggcgagggcagcacaaaggga

SEQ ID NO: 73 - DNA, 51 bp, Artificial Sequence
  linker
tctagcggcggaggcggatctggcgggggaggatctgggggaggcggctct

SEQ ID NO: 74 - DNA, 702 bp, Artificial Sequence
  spacer
cctgccgagcctaagagccccgacaagacccacacctgtcccccttgtcctgcccctccagtggctggccctagcgtgttcctgttccccccaaagcccaaggataccctgatgatcgcccggacccccgaagtcacatgcgtggtggtggacgtgagccacgaagaccctgaggtcaagttcaactggtacgtggacggcgtggaggtgcataatgccaagacaaagccgcgggaggagcagtacaacagcacgtaccgtgtggtcagcgtcctcaccgtcctgcaccaggactggctgaatggcaaggagtacaagtgcaaggtctccaacaaagccctcccagcccccatcgagaaaaccatctccaaagccaaagggcagccccgagaaccacaggtgtacaccctgcccccatcccgggatgagctgaccaagaaccaggtcagcctgacctgcctggtcaaaggcttctatcccagcgacatcgccgtggagtgggagagcaatgggcagccggagaacaactacaagaccacgcctcccgtgctggactccgacggctccttcttcctctacagcaagctcaccgtggacaagagcaggtggcagcaggggaacgtcttctcatgctccgtgatgcatgaggctctgcacaaccactacacgcagaagagcctctccctgtctccgggtaaaaaa

SEQ ID NO: 75 - DNA, 705 bp, Artificial Sequence
  spacer
cctgccgagcctaagagccccgacaagacccacacctgtcccccttgtcctgcccctccagtggctggccctagcgtgttcctgttccccccaaagcccaaggataccctgatgatcgcccggacccccgaagtcacatgcgtggtggtggacgtgagccacgaagaccctgaggtcaagttcaactggtacgtggacggcgtggaggtgcataatgccaagacaaagccgcgggaggagcagtacaacagcacgtaccgtgtggtcagcgtcctcaccgtcctgcaccaggactggctgaatggcaaggagtacaagtgcaaggtctccaacaaagccctcccagcccccatcgagaaaaccatctccaaagccaaagggcagccccgagaaccacaggtgtacaccctgcccccatcccgggatgagctgaccaagaaccaggtgtccctgacctgcctcgtgaagggcttctacccctccgatatcgccgtggaatgggagagcaatggccagcccgagaacaactacaagaccaccccccctgtgctggacagcgacggctcattcttcctgtacagcaagctgacagtggacaagagccggtggcagcagggcaacgtgttcagctgcagcgtgatgcacgaggctctgcacaaccactacacccagaagtccctgagcagcctgagcccaggcaagaag

SEQ ID NO: 76 - DNA, 687 bp, Artificial Sequence
  spacer
gagagcaagtacggccctccctgccccccttgccctgcccccgagttcgagggcggacccagcgtgttcctgttcccccccaagcccaaggacaccctgatgatcagccggacccccgaggtgacctgcgtggtggtggacgtgagccaggaagatcccgaggtccagttcaattggtacgtggacggcgtggaagtgcacaacgccaagaccaagcccagagaggaacagttcaacagcacctaccgggtggtgtctgtgctgaccgtgctgcaccaggactggctgaacggcaaagaatacaagtgcaaggtgtccaacaagggcctgcccagcagcatcgaaaagaccatcagcaaggccaagggccagcctcgcgagccccaggtgtacaccctgcctccctcccaggaagagatgaccaagaaccaggtgtccctgacctgcctggtgaagggcttctaccccagcgacatcgccgtggagtgggagagcaacggccagcctgagaacaactacaagaccacccctcccgtgctggacagcgacggcagcttcttcctctacagccggctgaccgtggacaagagccggtggcaggaaggcaacgtctttagctgcagcgtgatgcacgaggccctgcacaaccactacacccagaagagcctgagcctgtccctgggcaag

SEQ ID NO: 77 - DNA, 357 bp, Artificial Sequence
  spacer
gagagcaagtacggccctccctgccccccttgccctggccagcctcgcgagccccaggtgtacaccctgcctccctcccaggaagagatgaccaagaaccaggtgtccctgacctgcctggtgaagggcttctaccccagcgacatcgccgtggagtgggagagcaacggccagcctgagaacaactacaagaccacccctcccgtgctggacagcgacggcagcttcttcctctacagccggctgaccgtggacaagagccggtggcaggaaggcaacgtctttagctgcagcgtgatgcacgaggccctgcacaaccactacacccagaagagcctgagcctgtccctgggcaag

SEQ ID NO: 78 - DNA, 36 bp, Artificial Sequence
  spacer
gagagcaagtacggccctccctgccccccttgccct

SEQ ID NO: 79 - DNA, 72 bp, Artificial Sequence
  transmembrane
atctacatctgggcccctctggccggcacctgtggcgtgctgctgctgtctctcgtgatcacactgtactgc

SEQ ID NO: 80 - DNA, 81 bp, Artificial Sequence
  transmembrane
ttttgggtgctggtggtggttggtggagtcctggcttgctatagcttgctagtaacagtggcctttattattttctgggtg

SEQ ID NO: 81 - DNA, 126 bp, Artificial Sequence
  intracellular
aagcggggcagaaagaagctgctgtacatcttcaagcagcccttcatgcggcccgtgcagaccacccaggaagaggacggctgctcctgcagattccccgaggaagaagaaggcggctgcgagctg

SEQ ID NO: 82 - DNA, 123 bp, Artificial Sequence
  intracellular
aggagtaagaggagcaggctcctgcacagtgactacatgaacatgactccccgccgccccgggcccacccgcaagcattaccagccctatgccccaccacgcgacttcgcagcctatcgctcc

SEQ ID NO: 83 - DNA, 123 bp, Artificial Sequence
  intracellular
aggagtaagaggagcaggctcctgcacagtgactacatgaacatgactccccgtcgacccgggcccacccgcaagcattaccagccctatgccccaccacgcgacttcgcagcctatcgctcc

SEQ ID NO: 84 - DNA, 342 bp, Artificial Sequence
  intracellular
ctgagagtgaagttcagcaggagcgcagacgcccccgcgtaccagcagggccagaaccagctctataacgagctcaatctaggacgaagagaggagtacgatgttttggacaagagacgtggccgggaccctgagatggggggaaagccgagaaggaagaaccctcaggaaggcctgtacaatgaactgcagaaagataagatggcggaggcctacagtgagattgggatgaaaggcgagcgccggaggggcaaggggcacgatggcctttaccagggtctcagtacagccaccaaggacacctacgacgcccttcacatgcaggccctgccccctcgctga

SEQ ID NO: 85 - DNA, 339 bp, Artificial Sequence
  intracellular
ctgcgcgtgaagttttctagaagcgccgacgcccctgcctaccagcagggccagaaccagctgtacaacgagctgaacctgggcagacgggaagagtacgacgtgctggataagcggagaggccgggaccctgagatgggcggcaagcctagaagaaagaacccccaggaaggcctgtataacgaactgcagaaagacaagatggccgaggcctacagcgagatcggaatgaagggcgagcggagaagaggcaagggccacgatggactgtaccagggcctgagcaccgccaccaaggacacctatgacgccctgcacatgcaggctctgccccccaga

SEQ ID NO: 86 - DNA, 2055 bp, Artificial Sequence
  construct
atggatttccaggtgcagatcttcagcttcctgctgatctccgccagcgtgatcatgagccgcgaggtgcagctggtggaatctggcggaggactggtgcagcctggcggctctctgagactgtcttgtgccgccagcggcttcaccttcagccggtactggtttagctgggtgcgccaggcccctggcaagggactcgtgtgggtgggagagatcaaccccagcagcagcaccatcaactacgcccccagcctgaaggacaagttcaccatcagcagagacaacgccaagaacaccctgtacctgcagatgaacagcctgcgggccgaggacaccgccgtgtactattgtgccagcctgtactacgactacggcgacgcctacgattactggggccagggcacactggtgactgttagctccggcagcaccagcggctccggcaagcctggctctggcgagggcagcacaaagggagagatcgtgatgacacagagccctgccaccctgagcgtgtccccaggcgaaagagctaccctgagctgcaaggccagccagagcgtggaaagcaacgtggcctggtatcagcagaagcccggacaggctcctcgggccctgatctacagcgccagcctgagattcagcggcatccccgccaggtttagcggctctggcagcggcaccgagttcaccctgacaatcagcagcctgcagagcgaggactttgccgtgtattactgccagcagtacaacaactaccccctgaccttcggagccggcaccaagctggagctgaagcctgccgagcctaagagccccgacaagacccacacctgtcccccttgtcctgcccctccagtggctggccctagcgtgttcctgttccccccaaagcccaaggataccctgatgatcgcccggacccccgaagtcacatgcgtggtggtggacgtgagccacgaagaccctgaggtcaagttcaactggtacgtggacggcgtggaggtgcataatgccaagacaaagccgcgggaggagcagtacaacagcacgtaccgtgtggtcagcgtcctcaccgtcctgcaccaggactggctgaatggcaaggagtacaagtgcaaggtctccaacaaagccctcccagcccccatcgagaaaaccatctccaaagccaaagggcagccccgagaaccacaggtgtacaccctgcccccatcccgggatgagctgaccaagaaccaggtcagcctgacctgcctggtcaaaggcttctatcccagcgacatcgccgtggagtgggagagcaatgggcagccggagaacaactacaagaccacgcctcccgtgctggactccgacggctccttcttcctctacagcaagctcaccgtggacaagagcaggtggcagcaggggaacgtcttctcatgctccgtgatgcatgaggctctgcacaaccactacacgcagaagagcctctccctgtctccgggtaaaaaagatcccaaattttgggtgctggtggtggttggtggagtcctggcttgctatagcttgctagtaacagtggcctttattattttctgggtgaggagtaagaggagcaggctcctgcacagtgactacatgaacatgactccccgccgccccgggcccacccgcaagcattaccagccctatgccccaccacgcgacttcgcagcctatcgctccctgagagtgaagttcagcaggagcgcagacgcccccgcgtaccagcagggccagaaccagctctataacgagctcaatctaggacgaagagaggagtacgatgttttggacaagagacgtggccgggaccctgagatggggggaaagccgagaaggaagaaccctcaggaaggcctgtacaatgaactgcagaaagataagatggcggaggcctacagtgagattgggatgaaaggcgagcgccggaggggcaaggggcacgatggcctttaccagggtctcagtacagccaccaaggacacctacgacgcccttcacatgcaggccctgccccctcgctga

SEQ ID NO: 87 - DNA, 2055 bp, Artificial Sequence
  construct
atggatttccaggtgcagatcttcagcttcctgctgatctccgccagcgtgatcatgagccgcgagatcgtgatgacacagagccctgccaccctgagcgtgtccccaggcgaaagagctaccctgagctgcaaggccagccagagcgtggaaagcaacgtggcctggtatcagcagaagcccggacaggctcctcgggccctgatctacagcgccagcctgagattcagcggcatccccgccaggtttagcggctctggcagcggcaccgagttcaccctgacaatcagcagcctgcagagcgaggactttgccgtgtattactgccagcagtacaacaactaccccctgaccttcggagccggcaccaagctggagctgaagggcagcaccagcggctccggcaagcctggctctggcgagggcagcacaaagggagaggtgcagctggtggaatctggcggaggactggtgcagcctggcggctctctgagactgtcttgtgccgccagcggcttcaccttcagccggtactggtttagctgggtgcgccaggcccctggcaagggactcgtgtgggtgggagagatcaaccccagcagcagcaccatcaactacgcccccagcctgaaggacaagttcaccatcagcagagacaacgccaagaacaccctgtacctgcagatgaacagcctgcgggccgaggacaccgccgtgtactattgtgccagcctgtactacgactacggcgacgcctacgattactggggccagggcacactggtgactgttagctcccctgccgagcctaagagccccgacaagacccacacctgtcccccttgtcctgcccctccagtggctggccctagcgtgttcctgttccccccaaagcccaaggataccctgatgatcgcccggacccccgaagtcacatgcgtggtggtggacgtgagccacgaagaccctgaggtcaagttcaactggtacgtggacggcgtggaggtgcataatgccaagacaaagccgcgggaggagcagtacaacagcacgtaccgtgtggtcagcgtcctcaccgtcctgcaccaggactggctgaatggcaaggagtacaagtgcaaggtctccaacaaagccctcccagcccccatcgagaaaaccatctccaaagccaaagggcagccccgagaaccacaggtgtacaccctgcccccatcccgggatgagctgaccaagaaccaggtcagcctgacctgcctggtcaaaggcttctatcccagcgacatcgccgtggagtgggagagcaatgggcagccggagaacaactacaagaccacgcctcccgtgctggactccgacggctccttcttcctctacagcaagctcaccgtggacaagagcaggtggcagcaggggaacgtcttctcatgctccgtgatgcatgaggctctgcacaaccactacacgcagaagagcctctccctgtctccgggtaaaaaagatcccaaattttgggtgctggtggtggttggtggagtcctggcttgctatagcttgctagtaacagtggcctttattattttctgggtgaggagtaagaggagcaggctcctgcacagtgactacatgaacatgactccccgccgccccgggcccacccgcaagcattaccagccctatgccccaccacgcgacttcgcagcctatcgctccctgagagtgaagttcagcaggagcgcagacgcccccgcgtaccagcagggccagaaccagctctataacgagctcaatctaggacgaagagaggagtacgatgttttggacaagagacgtggccgggaccctgagatggggggaaagccgagaaggaagaaccctcaggaaggcctgtacaatgaactgcagaaagataagatggcggaggcctacagtgagattgggatgaaaggcgagcgccggaggggcaaggggcacgatggcctttaccagggtctcagtacagccaccaaggacacctacgacgcccttcacatgcaggccctgccccctcgctga

SEQ ID NO: 88 - DNA, 2055 bp, Artificial Sequence
  construct
atggatttccaggtgcagatcttcagcttcctgctgatctccgccagcgtgatcatgagccgcgaagtgcagctggtcgaatctggaggaggcctggttcagcctggtggcagccttaggctctcttgtgcagcctctggctttaccttctcacggtattggttcagctgggtgagacaggctccagggaaaggtctggtgtgggtaggggagataaaccccagcagcagcacgatcaactatgctccgtcactgaaagacaagttcaccatttcccgcgataatgccaagaacactctctacttgcagatgaattcccttcgagccgaggatacagcggtgtactactgcgccagtctgtactacgactatggggacgcatacgactattggggacaaggcacactggtgactgttagctccggcagcaccagcggctccggcaagcctggctctggcgagggcagcacaaagggagagatcgtgatgacccagtctcctgctaccctgagcgtttctcccggtgaaagggccacactcagctgcaaagcctctcaaagcgtggagagcaatgtcgcctggtatcagcagaaacctggccaagctccgagagcactgatctattccgcgtcattgcgcttttccggcataccagcacggtttagtggctcagggagtgggactgagttcactctgacgattagctcccttcagtcagaggatttcgccgtgtactactgtcagcagtacaacaactatcccctcacattcggagctggaaccaagctggaactgaagcctgccgagcctaagagccccgacaagacccacacctgtcccccttgtcctgcccctccagtggctggccctagcgtgttcctgttccccccaaagcccaaggataccctgatgatcgcccggacccccgaagtcacatgcgtggtggtggacgtgagccacgaagaccctgaggtcaagttcaactggtacgtggacggcgtggaggtgcataatgccaagacaaagccgcgggaggagcagtacaacagcacgtaccgtgtggtcagcgtcctcaccgtcctgcaccaggactggctgaatggcaaggagtacaagtgcaaggtctccaacaaagccctcccagcccccatcgagaaaaccatctccaaagccaaagggcagccccgagaaccacaggtgtacaccctgcccccatcccgggatgagctgaccaagaaccaggtcagcctgacctgcctggtcaaaggcttctatcccagcgacatcgccgtggagtgggagagcaatgggcagccggagaacaactacaagaccacgcctcccgtgctggactccgacggctccttcttcctctacagcaagctcaccgtggacaagagcaggtggcagcaggggaacgtcttctcatgctccgtgatgcatgaggctctgcacaaccactacacgcagaagagcctctccctgtctccgggtaaaaaagatcccaaattttgggtgctggtggtggttggtggagtcctggcttgctatagcttgctagtaacagtggcctttattattttctgggtgaggagtaagaggagcaggctcctgcacagtgactacatgaacatgactccccgccgccccgggcccacccgcaagcattaccagccctatgccccaccacgcgacttcgcagcctatcgctccctgagagtgaagttcagcaggagcgcagacgcccccgcgtaccagcagggccagaaccagctctataacgagctcaatctaggacgaagagaggagtacgatgttttggacaagagacgtggccgggaccctgagatggggggaaagccgagaaggaagaaccctcaggaaggcctgtacaatgaactgcagaaagataagatggcggaggcctacagtgagattgggatgaaaggcgagcgccggaggggcaaggggcacgatggcctttaccagggtctcagtacagccaccaaggacacctacgacgcccttcacatgcaggccctgccccctcgctga

SEQ ID NO: 89 - DNA, 2031 bp, Artificial Sequence
  construct
atggatttccaggtgcagatcttcagcttcctgctgatctccgccagcgtgatcatgagccgcgaggtgcagctggtggaatctggcggaggactggtgcagcctggcggctctctgagactgtcttgtgccgccagcggcttcaccttcagccggtactggtttagctgggtgcgccaggcccctggcaagggactcgtgtgggtgggagagatcaaccccagcagcagcaccatcaactacgcccccagcctgaaggacaagttcaccatcagcagagacaacgccaagaacaccctgtacctgcagatgaacagcctgcgggccgaggacaccgccgtgtactattgtgccagcctgtactacgactacggcgacgcctacgattactggggccagggcacactggtgactgttagctccggcagcaccagcggctccggcaagcctggctctggcgagggcagcacaaagggagagatcgtgatgacacagagccctgccaccctgagcgtgtccccaggcgaaagagctaccctgagctgcaaggccagccagagcgtggaaagcaacgtggcctggtatcagcagaagcccggacaggctcctcgggccctgatctacagcgccagcctgagattcagcggcatccccgccaggttttccggatctggcagcggcaccgagttcaccctgacaatcagcagcctgcagagcgaggactttgccgtgtattactgccagcagtacaacaactaccccctgaccttcggagccggcaccaagctggagctgaaggagagcaagtacggccctccctgccccccttgccctgcccccgagttcgagggcggacccagcgtgttcctgttcccccccaagcccaaggacaccctgatgatcagccggacccccgaggtgacctgcgtggtggtggacgtgagccaggaagatcccgaggtccagttcaattggtacgtggacggcgtggaagtgcacaacgccaagaccaagcccagagaggaacagttcaacagcacctaccgggtggtgtctgtgctgaccgtgctgcaccaggactggctgaacggcaaagaatacaagtgcaaggtgtccaacaagggcctgcccagcagcatcgaaaagaccatcagcaaggccaagggccagcctcgcgagccccaggtgtacaccctgcctccctcccaggaagagatgaccaagaaccaggtgtccctgacctgcctggtgaagggcttctaccccagcgacatcgccgtggagtgggagagcaacggccagcctgagaacaactacaagaccacccctcccgtgctggacagcgacggcagcttcttcctctacagccggctgaccgtggacaagagccggtggcaggaaggcaacgtctttagctgcagcgtgatgcacgaggccctgcacaaccactacacccagaagagcctgagcctgtccctgggcaagttttgggtgctggtggtggttggtggagtcctggcttgctatagcttgctagtaacagtggcctttattattttctgggtgaggagtaagaggagcaggctcctgcacagtgactacatgaacatgactccccgtcgacccgggcccacccgcaagcattaccagccctatgccccaccacgcgacttcgcagcctatcgctccctgagagtgaagttcagcaggagcgcagacgcccccgcgtaccagcagggccagaaccagctctataacgagctcaatctaggacgaagagaggagtacgatgttttggacaagagacgtggccgggaccctgagatggggggaaagccgagaaggaagaaccctcaggaaggcctgtacaatgaactgcagaaagataagatggcggaggcctacagtgagattgggatgaaaggcgagcgccggaggggcaaggggcacgatggcctttaccagggtctcagtacagccaccaaggacacctacgacgcccttcacatgcaggccctgccccctcgctga

SEQ ID NO: 90 - DNA, 1701 bp, Artificial Sequence
  construct
atggatttccaggtgcagatcttcagcttcctgctgatctccgccagcgtgatcatgagccgcgaggtgcagctggtggaatctggcggaggactggtgcagcctggcggctctctgagactgtcttgtgccgccagcggcttcaccttcagccggtactggtttagctgggtgcgccaggcccctggcaagggactcgtgtgggtgggagagatcaaccccagcagcagcaccatcaactacgcccccagcctgaaggacaagttcaccatcagcagagacaacgccaagaacaccctgtacctgcagatgaacagcctgcgggccgaggacaccgccgtgtactattgtgccagcctgtactacgactacggcgacgcctacgattactggggccagggcacactggtgactgttagctccggcagcaccagcggctccggcaagcctggctctggcgagggcagcacaaagggagagatcgtgatgacacagagccctgccaccctgagcgtgtccccaggcgaaagagctaccctgagctgcaaggccagccagagcgtggaaagcaacgtggcctggtatcagcagaagcccggacaggctcctcgggccctgatctacagcgccagcctgagattcagcggcatccccgccaggttttccggatctggcagcggcaccgagttcaccctgacaatcagcagcctgcagagcgaggactttgccgtgtattactgccagcagtacaacaactaccccctgaccttcggagccggcaccaagctggagctgaaggagagcaagtacggccctccctgccccccttgccctggccagcctcgcgagccccaggtgtacaccctgcctccctcccaggaagagatgaccaagaaccaggtgtccctgacctgcctggtgaagggcttctaccccagcgacatcgccgtggagtgggagagcaacggccagcctgagaacaactacaagaccacccctcccgtgctggacagcgacggcagcttcttcctctacagccggctgaccgtggacaagagccggtggcaggaaggcaacgtctttagctgcagcgtgatgcacgaggccctgcacaaccactacacccagaagagcctgagcctgtccctgggcaagttttgggtgctggtggtggttggtggagtcctggcttgctatagcttgctagtaacagtggcctttattattttctgggtgaggagtaagaggagcaggctcctgcacagtgactacatgaacatgactccccgtcgacccgggcccacccgcaagcattaccagccctatgccccaccacgcgacttcgcagcctatcgctccctgagagtgaagttcagcaggagcgcagacgcccccgcgtaccagcagggccagaaccagctctataacgagctcaatctaggacgaagagaggagtacgatgttttggacaagagacgtggccgggaccctgagatggggggaaagccgagaaggaagaaccctcaggaaggcctgtacaatgaactgcagaaagataagatggcggaggcctacagtgagattgggatgaaaggcgagcgccggaggggcaaggggcacgatggcctttaccagggtctcagtacagccaccaaggacacctacgacgcccttcacatgcaggccctgccccctcgctga

SEQ ID NO: 91 - DNA, 1380 bp, Artificial Sequence
  construct
atggatttccaggtgcagatcttcagcttcctgctgatctccgccagcgtgatcatgagccgcgaggtgcagctggtggaatctggcggaggactggtgcagcctggcggctctctgagactgtcttgtgccgccagcggcttcaccttcagccggtactggtttagctgggtgcgccaggcccctggcaagggactcgtgtgggtgggagagatcaaccccagcagcagcaccatcaactacgcccccagcctgaaggacaagttcaccatcagcagagacaacgccaagaacaccctgtacctgcagatgaacagcctgcgggccgaggacaccgccgtgtactattgtgccagcctgtactacgactacggcgacgcctacgattactggggccagggcacactggtgactgttagctccggcagcaccagcggctccggcaagcctggctctggcgagggcagcacaaagggagagatcgtgatgacacagagccctgccaccctgagcgtgtccccaggcgaaagagctaccctgagctgcaaggccagccagagcgtggaaagcaacgtggcctggtatcagcagaagcccggacaggctcctcgggccctgatctacagcgccagcctgagattcagcggcatccccgccaggttttccggatctggcagcggcaccgagttcaccctgacaatcagcagcctgcagagcgaggactttgccgtgtattactgccagcagtacaacaactaccccctgaccttcggagccggcaccaagctggagctgaaggagagcaagtacggccctccctgccccccttgccctttttgggtgctggtggtggttggtggagtcctggcttgctatagcttgctagtaacagtggcctttattattttctgggtgaggagtaagaggagcaggctcctgcacagtgactacatgaacatgactccccgtcgacccgggcccacccgcaagcattaccagccctatgccccaccacgcgacttcgcagcctatcgctccctgagagtgaagttcagcaggagcgcagacgcccccgcgtaccagcagggccagaaccagctctataacgagctcaatctaggacgaagagaggagtacgatgttttggacaagagacgtggccgggaccctgagatggggggaaagccgagaaggaagaaccctcaggaaggcctgtacaatgaactgcagaaagataagatggcggaggcctacagtgagattgggatgaaaggcgagcgccggaggggcaaggggcacgatggcctttaccagggtctcagtacagccaccaaggacacctacgacgcccttcacatgcaggccctgccccctcgctga

SEQ ID NO: 92 - DNA, 2040 bp, Artificial Sequence
  construct
atggatttccaggtgcagatcttcagcttcctgctgatctccgccagcgtgatcatgagccgcgaggtgcagctggtggaatctggcggaggactggtgcagcctggcggctctctgagactgtcttgtgccgccagcggcttcaccttcagccggtactggtttagctgggtgcgccaggcccctggcaagggactcgtgtgggtgggagagatcaaccccagcagcagcaccatcaactacgcccccagcctgaaggacaagttcaccatcagcagagacaacgccaagaacaccctgtacctgcagatgaacagcctgcgggccgaggacaccgccgtgtactattgtgccagcctgtactacgactacggcgacgcctacgattactggggccagggcacactggtgactgttagctccggcagcaccagcggctccggcaagcctggctctggcgagggcagcacaaagggagagatcgtgatgacacagagccctgccaccctgagcgtgtccccaggcgaaagagctaccctgagctgcaaggccagccagagcgtggaaagcaacgtggcctggtatcagcagaagcccggacaggctcctcgggccctgatctacagcgccagcctgagattcagcggcatccccgccaggtttagcggctctggcagcggcaccgagttcaccctgacaatcagcagcctgcagagcgaggactttgccgtgtattactgccagcagtacaacaactaccccctgaccttcggagccggcaccaagctggagctgaagcctgccgagcctaagagccccgacaagacccacacctgtcccccttgtcctgcccctccagtggctggccctagcgtgttcctgttccccccaaagcccaaggataccctgatgatcgcccggacccccgaagtcacatgcgtggtggtggacgtgagccacgaagaccctgaggtcaagttcaactggtacgtggacggcgtggaggtgcataatgccaagacaaagccgcgggaggagcagtacaacagcacgtaccgtgtggtcagcgtcctcaccgtcctgcaccaggactggctgaatggcaaggagtacaagtgcaaggtctccaacaaagccctcccagcccccatcgagaaaaccatctccaaagccaaagggcagccccgagaaccacaggtgtacaccctgcccccatcccgggatgagctgaccaagaaccaggtgtccctgacctgcctcgtgaagggcttctacccctccgatatcgccgtggaatgggagagcaatggccagcccgagaacaactacaagaccaccccccctgtgctggacagcgacggctcattcttcctgtacagcaagctgacagtggacaagagccggtggcagcagggcaacgtgttcagctgcagcgtgatgcacgaggctctgcacaaccactacacccagaagtccctgagcagcctgagcccaggcaagaagatctacatctgggcccctctggccggcacctgtggcgtgctgctgctgtctctcgtgatcacactgtactgcaagcggggcagaaagaagctgctgtacatcttcaagcagcccttcatgcggcccgtgcagaccacccaggaagaggacggctgctcctgcagattccccgaggaagaagaaggcggctgcgagctgctgcgcgtgaagttttctagaagcgccgacgcccctgcctaccagcagggccagaaccagctgtacaacgagctgaacctgggcagacgggaagagtacgacgtgctggataagcggagaggccgggaccctgagatgggcggcaagcctagaagaaagaacccccaggaaggcctgtataacgaactgcagaaagacaagatggccgaggcctacagcgagatcggaatgaagggcgagcggagaagaggcaagggccacgatggactgtaccagggcctgagcaccgccaccaaggacacctatgacgccctgcacatgcaggctctgccccccaga

SEQ ID NO: 93 - DNA, 2040 bp, Artificial Sequence
  construct
atggatttccaggtgcagatcttcagcttcctgctgatctccgccagcgtgatcatgagccgcgagatcgtgatgacacagagccctgccaccctgagcgtgtccccaggcgaaagagctaccctgagctgcaaggccagccagagcgtggaaagcaacgtggcctggtatcagcagaagcccggacaggctcctcgggccctgatctacagcgccagcctgagattcagcggcatccccgccaggtttagcggctctggcagcggcaccgagttcaccctgacaatcagcagcctgcagagcgaggactttgccgtgtattactgccagcagtacaacaactaccccctgaccttcggagccggcaccaagctggagctgaagggcagcaccagcggctccggcaagcctggctctggcgagggcagcacaaagggagaggtgcagctggtggaatctggcggaggactggtgcagcctggcggctctctgagactgtcttgtgccgccagcggcttcaccttcagccggtactggtttagctgggtgcgccaggcccctggcaagggactcgtgtgggtgggagagatcaaccccagcagcagcaccatcaactacgcccccagcctgaaggacaagttcaccatcagcagagacaacgccaagaacaccctgtacctgcagatgaacagcctgcgggccgaggacaccgccgtgtactattgtgccagcctgtactacgactacggcgacgcctacgattactggggccagggcacactggtgactgttagctcccctgccgagcctaagagccccgacaagacccacacctgtcccccttgtcctgcccctccagtggctggccctagcgtgttcctgttccccccaaagcccaaggataccctgatgatcgcccggacccccgaagtcacatgcgtggtggtggacgtgagccacgaagaccctgaggtcaagttcaactggtacgtggacggcgtggaggtgcataatgccaagacaaagccgcgggaggagcagtacaacagcacgtaccgtgtggtcagcgtcctcaccgtcctgcaccaggactggctgaatggcaaggagtacaagtgcaaggtctccaacaaagccctcccagcccccatcgagaaaaccatctccaaagccaaagggcagccccgagaaccacaggtgtacaccctgcccccatcccgggatgagctgaccaagaaccaggtgtccctgacctgcctcgtgaagggcttctacccctccgatatcgccgtggaatgggagagcaatggccagcccgagaacaactacaagaccaccccccctgtgctggacagcgacggctcattcttcctgtacagcaagctgacagtggacaagagccggtggcagcagggcaacgtgttcagctgcagcgtgatgcacgaggctctgcacaaccactacacccagaagtccctgagcagcctgagcccaggcaagaagatctacatctgggcccctctggccggcacctgtggcgtgctgctgctgtctctcgtgatcacactgtactgcaagcggggcagaaagaagctgctgtacatcttcaagcagcccttcatgcggcccgtgcagaccacccaggaagaggacggctgctcctgcagattccccgaggaagaagaaggcggctgcgagctgctgcgcgtgaagttttctagaagcgccgacgcccctgcctaccagcagggccagaaccagctgtacaacgagctgaacctgggcagacgggaagagtacgacgtgctggataagcggagaggccgggaccctgagatgggcggcaagcctagaagaaagaacccccaggaaggcctgtataacgaactgcagaaagacaagatggccgaggcctacagcgagatcggaatgaagggcgagcggagaagaggcaagggccacgatggactgtaccagggcctgagcaccgccaccaaggacacctatgacgccctgcacatgcaggctctgccccccaga

SEQ ID NO: 94 - DNA, 2040 bp, Artificial Sequence
  construct
atggatttccaggtgcagatcttcagcttcctgctgatctccgccagcgtgatcatgagccgcgaagtgcagctggtcgaatctggaggaggcctggttcagcctggtggcagccttaggctctcttgtgcagcctctggctttaccttctcacggtattggttcagctgggtgagacaggctccagggaaaggtctggtgtgggtaggggagataaaccccagcagcagcacgatcaactatgctccgtcactgaaagacaagttcaccatttcccgcgataatgccaagaacactctctacttgcagatgaattcccttcgagccgaggatacagcggtgtactactgcgccagtctgtactacgactatggggacgcatacgactattggggacaaggcacactggtgactgttagctccggcagcaccagcggctccggcaagcctggctctggcgagggcagcacaaagggagagatcgtgatgacccagtctcctgctaccctgagcgtttctcccggtgaaagggccacactcagctgcaaagcctctcaaagcgtggagagcaatgtcgcctggtatcagcagaaacctggccaagctccgagagcactgatctattccgcgtcattgcgcttttccggcataccagcacggtttagtggctcagggagtgggactgagttcactctgacgattagctcccttcagtcagaggatttcgccgtgtactactgtcagcagtacaacaactatcccctcacattcggagctggaaccaagctggaactgaagcctgccgagcctaagagccccgacaagacccacacctgtcccccttgtcctgcccctccagtggctggccctagcgtgttcctgttccccccaaagcccaaggataccctgatgatcgcccggacccccgaagtcacatgcgtggtggtggacgtgagccacgaagaccctgaggtcaagttcaactggtacgtggacggcgtggaggtgcataatgccaagacaaagccgcgggaggagcagtacaacagcacgtaccgtgtggtcagcgtcctcaccgtcctgcaccaggactggctgaatggcaaggagtacaagtgcaaggtctccaacaaagccctcccagcccccatcgagaaaaccatctccaaagccaaagggcagccccgagaaccacaggtgtacaccctgcccccatcccgggatgagctgaccaagaaccaggtgtccctgacctgcctcgtgaagggcttctacccctccgatatcgccgtggaatgggagagcaatggccagcccgagaacaactacaagaccaccccccctgtgctggacagcgacggctcattcttcctgtacagcaagctgacagtggacaagagccggtggcagcagggcaacgtgttcagctgcagcgtgatgcacgaggctctgcacaaccactacacccagaagtccctgagcagcctgagcccaggcaagaagatctacatctgggcccctctggccggcacctgtggcgtgctgctgctgtctctcgtgatcacactgtactgcaagcggggcagaaagaagctgctgtacatcttcaagcagcccttcatgcggcccgtgcagaccacccaggaagaggacggctgctcctgcagattccccgaggaagaagaaggcggctgcgagctgctgcgcgtgaagttttctagaagcgccgacgcccctgcctaccagcagggccagaaccagctgtacaacgagctgaacctgggcagacgggaagagtacgacgtgctggataagcggagaggccgggaccctgagatgggcggcaagcctagaagaaagaacccccaggaaggcctgtataacgaactgcagaaagacaagatggccgaggcctacagcgagatcggaatgaagggcgagcggagaagaggcaagggccacgatggactgtaccagggcctgagcaccgccaccaaggacacctatgacgccctgcacatgcaggctctgccccccaga